European Patent Application EP 4 116 436 A1, published January 11, 2023. Title: Method and System for Screening Neoantigens, and Use thereof. Applicant: Korea Advanced Institute of Science and Technology PentaMedix Co., Ltd. The sequence listing filed with the application follows.

SEQUENCE LISTING (65 sequences)

SEQ ID NO: 1 - protein, 9 aa, Artificial Sequence
  Neoantigen_HLA-A02 binding
RLWHLLLQV

SEQ ID NO: 2 - protein, 9 aa, Artificial Sequence
  Neoantigen_HLA-A02 binding
LMFSRCTSV

SEQ ID NO: 3 - protein, 9 aa, Artificial Sequence
  Neoantigen_HLA-A02 binding
RLLDEYNLV

SEQ ID NO: 4 - protein, 9 aa, Artificial Sequence
  Neoantigen_HLA-A02 binding
LLALWLCWA

SEQ ID NO: 5 - protein, 9 aa, Artificial Sequence
  Neoantigen_HLA-A02 binding
HLYPGPCHL

SEQ ID NO: 6 - protein, 9 aa, Artificial Sequence
  Neoantigen_HLA-A02 binding
RLMTHYCAM

SEQ ID NO: 7 - protein, 9 aa, Artificial Sequence
  Neoantigen_HLA-A02 binding
GLLPLASTV

SEQ ID NO: 8 - protein, 9 aa, Artificial Sequence
  Neoantigen_HLA-A02 binding
FLLGFLHSG

SEQ ID NO: 9 - protein, 9 aa, Artificial Sequence
  Neoantigen_HLA-A02 binding
LMNSLVSQV

SEQ ID NO: 10 - protein, 9 aa, Artificial Sequence
  Neoantigen_HLA-A02 binding
CLYAFECKI

SEQ ID NO: 11 - protein, 9 aa, Artificial Sequence
  Neoantigen_HLA-A02 binding
KTFPVQLWV

SEQ ID NO: 12 - protein, 9 aa, Artificial Sequence
  Neoantigen_HLA-A02 binding
GLLAESTWA

SEQ ID NO: 13 - protein, 9 aa, Artificial Sequence
  Neoantigen_HLA-A02 binding
SMQNHIPQV

SEQ ID NO: 14 - protein, 9 aa, Artificial Sequence
  Neoantigen_HLA-A02 binding
CQLAKTCPV

SEQ ID NO: 15 - protein, 9 aa, Artificial Sequence
  Neoantigen_HLA-A02 binding
LLGPNSFEV

SEQ ID NO: 16 - protein, 9 aa, Artificial Sequence
  Neoantigen_HLA-A02 binding
SLSYWRASV

SEQ ID NO: 17 - protein, 9 aa, Artificial Sequence
  Neoantigen_HLA-A02 binding
RVAQYPFEV

SEQ ID NO: 18 - protein, 9 aa, Artificial Sequence
  Neoantigen_HLA-A02 binding
LLAETCWNG

SEQ ID NO: 19 - protein, 9 aa, Artificial Sequence
  Neoantigen_HLA-A02 binding
VLQPAPHQV

SEQ ID NO: 20 - protein, 9 aa, Artificial Sequence
  Neoantigen_HLA-A02 binding
YLHCEWATI

SEQ ID NO: 21 - protein, 9 aa, Artificial Sequence
  Neoantigen_HLA-A02 binding
LLAESTWAL

SEQ ID NO: 22 - protein, 9 aa, Artificial Sequence
  Neoantigen_HLA-A02 binding
PLEEWNQWV

SEQ ID NO: 23 - protein, 9 aa, Artificial Sequence
  Neoantigen_HLA-A02 binding
ALNEMFCQL

SEQ ID NO: 24 - protein, 9 aa, Artificial Sequence
  Neoantigen_HLA-A02 binding
LLRRNSFEV

SEQ ID NO: 25 - protein, 9 aa, Artificial Sequence
  Neoantigen_HLA-A02 binding
ALPQHLIRV

SEQ ID NO: 26 - protein, 9 aa, Artificial Sequence
  Neoantigen_HLA-A02 binding
MAGGWVAHL

SEQ ID NO: 27 - protein, 9 aa, Artificial Sequence
  Neoantigen_HLA-A02 binding
GLNSFEVRV

SEQ ID NO: 28 - protein, 9 aa, Artificial Sequence
  Neoantigen_HLA-A02 binding
CQLAKTFPV

SEQ ID NO: 29 - protein, 9 aa, Artificial Sequence
  Neoantigen_HLA-A02 binding
NMANMPPQV

SEQ ID NO: 30 - protein, 9 aa, Artificial Sequence
  Neoantigen_HLA-A02 binding
YTEAEEFFV

SEQ ID NO: 31 - protein, 9 aa, Artificial Sequence
  Neoantigen_HLA-A02 binding
TLMSVPRYL

SEQ ID NO: 32 - protein, 9 aa, Artificial Sequence
  Neoantigen_HLA-A02 binding
KMWVDRYLA

SEQ ID NO: 33 - protein, 9 aa, Artificial Sequence
  Neoantigen_HLA-A02 binding
GLAPPQYLI

SEQ ID NO: 34 - protein, 9 aa, Artificial Sequence
  Neoantigen_HLA-A02 binding
FLINSSYPG

SEQ ID NO: 35 - protein, 9 aa, Artificial Sequence
  Neoantigen_HLA-A02 binding
FMYFEFPQL

SEQ ID NO: 36 - protein, 9 aa, Artificial Sequence
  Neoantigen_HLA-A02 binding
AAFVLLFFV

SEQ ID NO: 37 - protein, 9 aa, Artificial Sequence
  Neoantigen_HLA-A02 binding
ILHVAVTNV

SEQ ID NO: 38 - protein, 9 aa, Artificial Sequence
  Neoantigen_HLA-A02 binding
RLRSRTCLL

SEQ ID NO: 39 - protein, 9 aa, Artificial Sequence
  Neoantigen_HLA-A02 binding
ALDTINILL

SEQ ID NO: 40 - protein, 9 aa, Artificial Sequence
  Neoantigen_HLA-A02 binding
LIYQMAPAV

SEQ ID NO: 41 - protein, 9 aa, Artificial Sequence
  Neoantigen_HLA-A02 binding
SQLPGLLEL

SEQ ID NO: 42 - protein, 9 aa, Artificial Sequence
  Neoantigen_HLA-A02 binding
CQLAKTYPV

SEQ ID NO: 43 - protein, 9 aa, Artificial Sequence
  Neoantigen_HLA-A02 binding
GMGPPMPTV

SEQ ID NO: 44 - protein, 9 aa, Artificial Sequence
  Neoantigen_HLA-A02 binding
FTINRNTGV

SEQ ID NO: 45 - protein, 9 aa, Artificial Sequence
  Neoantigen_HLA-A02 binding
LMDGRDVFL

SEQ ID NO: 46 - protein, 9 aa, Artificial Sequence
  Neoantigen_HLA-A02 binding
PLIEEACEL

SEQ ID NO: 47 - protein, 9 aa, Artificial Sequence
  Neoantigen_HLA-A02 binding
TMYQQQQQV

SEQ ID NO: 48 - protein, 9 aa, Artificial Sequence
  Neoantigen_HLA-A02 binding
SALHWAAAV

SEQ ID NO: 49 - protein, 9 aa, Artificial Sequence
  Neoantigen_HLA-A02 binding
RMHDGTTPL

SEQ ID NO: 50 - protein, 9 aa, Artificial Sequence
  Neoantigen_HLA-A02 binding
LLMENSIGG

SEQ ID NO: 51 - protein, 15 aa, Artificial Sequence
  Twistnb
TVVEEVVEKTPKKKK

SEQ ID NO: 52 - protein, 15 aa, Artificial Sequence
  Las1l
STGKAPYTLDTLHED

SEQ ID NO: 53 - protein, 15 aa, Artificial Sequence
  Irx1
ALPERDLVTRPDWPP

SEQ ID NO: 54 - protein, 15 aa, Artificial Sequence
  Muc5b
GATTMSVNISTIGTN

SEQ ID NO: 55 - protein, 15 aa, Artificial Sequence
  Smarca5
LGKTLQTISLLGYRK

SEQ ID NO: 56 - protein, 15 aa, Artificial Sequence
  Eri1
YDYICIIDFEATCKE

SEQ ID NO: 57 - protein, 15 aa, Artificial Sequence
  Tph2
FVKSITRPFSVYFNR

SEQ ID NO: 58 - protein, 9 aa, Artificial Sequence
  Eef2
RAPAGAAAG

SEQ ID NO: 59 - protein, 15 aa, Artificial Sequence
  Ssrp1
GRGDSSERDKSKKKK

SEQ ID NO: 60 - protein, 15 aa, Artificial Sequence
  Oas1g
GKSDADLVVFLNNLT

SEQ ID NO: 61 - protein, 15 aa, Artificial Sequence
  Gm15557
SRHSCAEFVKFRKSF

SEQ ID NO: 62 - protein, 15 aa, Artificial Sequence
  Ppp1cc
SFTSGAEVVAKFLHK

SEQ ID NO: 63 - protein, 15 aa, Artificial Sequence
  Pdcd6ip
TVGTRSLIMLAQAQE

SEQ ID NO: 64 - protein, 15 aa, Artificial Sequence
  Dync1h1
PTAPSVPIIDYEVSI

SEQ ID NO: 65 - protein, 15 aa, Artificial Sequence
  Eef2
SGVCVQTEIVLRQAI